European Patent Application EP 4 509 134 A1, published February 19, 2025. Title: COMPOSITION INCLUDING IL-32THETA MUTANT AND USE THEREOF. Applicant: KONKUK UNIVERSITY INDUSTRIAL COOPERATION CORP. The sequence listing filed with the application follows.

SEQUENCE LISTING (34 sequences)

SEQ ID NO: 1 - protein, 168 aa, synthetic construct
  REGION 1..168: note = IL-32theta mutant_amino acid seqence
MCFPKVLSDDMKKLKARMHQAIERFYDKMQNAESGRGQVMSSLAELEELTPLLEKERDGLRCRGNRSPVPDVEDPATEEPGESFCDKVMRWFQVMLQRLQTWWHGVLAWVKEKVVALVHAVQALWKQFQSFCCSLSELFMSSFQSYGAPRGDKEELTPQKCSEPQSSK

SEQ ID NO: 2 - DNA, 507 bp, synthetic construct
  misc_feature 1..507: note = IL-32theta mutant_nucleotide sequence
  source 1..507: mol_type = other DNA
atgtgcttcccgaaggtcctctctgatgacatgaagaagctgaaggcccgaatgcaccaggccatagaaagattttatgataaaatgcaaaatgcagaatcaggacgtggacaggtgatgtcgagcctggcagagctggaggagctcactcctctacttgaaaaagaaagagatggattacggtgccgaggcaacagatcccctgtcccggatgttgaggatcccgcaaccgaggagcctggggagagcttttgtgacaaggtcatgagatggttccaggtcatgctgcagcggctgcagacctggtggcacggggttctggcctgggtgaaggagaaggtggtggccctggtccatgcagtgcaggccctctggaaacagttccagagtttctgctgctctctgtcagagctcttcatgtcctctttccagtcctacggagccccacggggggacaaggaggagctgacaccccagaagtgctctgaaccccaatcctcaaaatga

SEQ ID NO: 3 - DNA, 504 bp, synthetic construct
  misc_feature 1..504: note = IL-32theta mutant_recombinant nucleotide sequence
  source 1..504: mol_type = other DNA
atgtgctttccgaaagtcctctctgatgacatgaaaaagcttaaagcgcgaatgcaccaggcgattgaaagattctatgataaaatgcagaatgcagaatcaggacgtggtcaggtgatgtcgagcctggcagaactggaggaacttactcctctacttgaaaaagaacgtgatggattacggtgccgcggtaaccgtagccctgttccggatgttgaagatccggcgaccgaggagccgggcgaaagcttttgtgacaaagttatgcgttggtttcaagttatgctgcaacgcctgcagacgtggaggcatggggttttagcatgggtgaaagaaaaggtagtagccctggtccatgctgtgcaggctttatggaagcagtttcaaagtttttgttgctctctgtcagaattgttcatgtcctctttccagtcatacggcgccccacgcggtgataaagaagaattgacaccacagaaatgtagtgaaccccaatccagtaaa

SEQ ID NO: 4 - DNA, 507 bp, synthetic construct
  misc_feature 1..507: note = IL-32theta wildtype
  source 1..507: mol_type = other DNA
atgtgcttcccgaaggtcctctctgatgacatgaagaagctgaaggcccgaatgcaccaggccatagaaagattttatgataaaatgcaaaatgcagaatcaggacgtggacaggtgatgtcgagcctggcagagctggaggagctcactcctctacttgaaaaagaaagagatggattacggtgccgaggcaacagatcccctgtcccggatgttgaggatcccgcaaccgaggagcctggggagagcttttgtgacaaggtcatgagatggttccaggccatgctgcagcggctgcagacctggtggcacggggttctggcctgggtgaaggagaaggtggtggccctggtccatgcagtgcaggccctctggaaacagttccagagtttctgctgctctctgtcagagctcttcatgtcctctttccagtcctacggagccccacggggggacaaggaggagctgacaccccagaagtgctctgaaccccaatcctcaaaatga

SEQ ID NO: 5 - DNA, 20 bp, synthetic construct
  source 1..20: mol_type = other DNA
agaacatcatccctgcctct

SEQ ID NO: 6 - DNA, 20 bp, synthetic construct
  source 1..20: mol_type = other DNA
ctgcttcaccaccttcttga

SEQ ID NO: 7 - DNA, 20 bp, synthetic construct
  source 1..20: mol_type = other DNA
acgtggacaggtgatgtcga

SEQ ID NO: 8 - DNA, 20 bp, synthetic construct
  source 1..20: mol_type = other DNA
gagcagcagaaactctggaa

SEQ ID NO: 9 - DNA, 22 bp, synthetic construct
  source 1..22: mol_type = other DNA
cgacagaccttccaggagaatc

SEQ ID NO: 10 - DNA, 23 bp, synthetic construct
  source 1..23: mol_type = other DNA
gtgcagttcagtgatcgtacacc

SEQ ID NO: 11 - DNA, 22 bp, synthetic construct
  source 1..22: mol_type = other DNA
agacagccactcacctcttcag

SEQ ID NO: 12 - DNA, 22 bp, synthetic construct
  source 1..22: mol_type = other DNA
ttctgccagtgcctctttgctg

SEQ ID NO: 13 - DNA, 20 bp, synthetic construct
  source 1..20: mol_type = other DNA
ggtctgtgtgaaggtgcagt

SEQ ID NO: 14 - DNA, 20 bp, synthetic construct
  source 1..20: mol_type = other DNA
gttttccttggggtccagac

SEQ ID NO: 15 - DNA, 22 bp, synthetic construct
  source 1..22: mol_type = other DNA
cggtgaaactctggctagacag

SEQ ID NO: 16 - DNA, 22 bp, synthetic construct
  source 1..22: mol_type = other DNA
gcaaaccgtagatgctcaggga

SEQ ID NO: 17 - DNA, 23 bp, synthetic construct
  source 1..23: mol_type = other DNA
cctccagagtttactgccatgac

SEQ ID NO: 18 - DNA, 22 bp, synthetic construct
  source 1..22: mol_type = other DNA
gtaggatctccgccactgattc

SEQ ID NO: 19 - DNA, 22 bp, synthetic construct
  source 1..22: mol_type = other DNA
aggcaaagcaggagtccactga

SEQ ID NO: 20 - DNA, 22 bp, synthetic construct
  source 1..22: mol_type = other DNA
atctggcgttccagggactcat

SEQ ID NO: 21 - DNA, 24 bp, synthetic construct
  source 1..24: mol_type = other DNA
caagtaatgtcgataaagaggagg

SEQ ID NO: 22 - DNA, 22 bp, synthetic construct
  source 1..22: mol_type = other DNA
gtgtcaccgttgaagagagtgg

SEQ ID NO: 23 - DNA, 22 bp, synthetic construct
  source 1..22: mol_type = other DNA
atggatgcctctgctctcactg

SEQ ID NO: 24 - DNA, 22 bp, synthetic construct
  source 1..22: mol_type = other DNA
cccgatgagaatggcagaaagc

SEQ ID NO: 25 - DNA, 22 bp, synthetic construct
  source 1..22: mol_type = other DNA
aggagaaggtgcctacgaagct

SEQ ID NO: 26 - DNA, 23 bp, synthetic construct
  source 1..23: mol_type = other DNA
gcacaggaaagtcttgctaaggc

SEQ ID NO: 27 - DNA, 23 bp, synthetic construct
  source 1..23: mol_type = other DNA
catggattccagcaatgtcctcc

SEQ ID NO: 28 - DNA, 22 bp, synthetic construct
  source 1..22: mol_type = other DNA
ttgaggcaggtggcattgaagg

SEQ ID NO: 29 - DNA, 22 bp, synthetic construct
  source 1..22: mol_type = other DNA
tctcctgcgtgagacacaaagg

SEQ ID NO: 30 - DNA, 22 bp, synthetic construct
  source 1..22: mol_type = other DNA
gagcactccatcttcagagacg

SEQ ID NO: 31 - DNA, 22 bp, synthetic construct
  source 1..22: mol_type = other DNA
agcggctgacgtgtgcagtaat

SEQ ID NO: 32 - DNA, 22 bp, synthetic construct
  source 1..22: mol_type = other DNA
tctgagacctctggcttcgtca

SEQ ID NO: 33 - DNA, 22 bp, synthetic construct
  source 1..22: mol_type = other DNA
gattctgtgcccacagtaaggc

SEQ ID NO: 34 - DNA, 22 bp, synthetic construct
  source 1..22: mol_type = other DNA
tggtcacagagccaccttcttg